European Patent Specification EP 3 551 653 B1, published November 1, 2023. Title: T cell receptors with improved pairing. Applicant: Immatics Biotechnologies GmbH. The sequence listing filed with the application follows.

SEQUENCE LISTING (4 sequences)

SEQ ID NO: 1 - protein, 92 aa, Artificial
  TCR alpha chain variable domain of R7P1D5 (TRAV5)
GEDVEQSLFLSVREGDSSVINCTYTDSSSTYLYWYKQEPGAGLQLLTYIFSINMDMKQDQRLTVLLNKKDKHLSLRIADTQTGDSAIYFCAE

SEQ ID NO: 2 - protein, 94 aa, Artificial
  TCR beta chain variable domain of R7P1D5 (TRBV12-4)
DAGVIQSPRHEVTEMGQEVTLRCKPISGHDYLFWYRQTMMRGLELLIYFNNNVPIDDSGMPEDRFSAKMPNASFSTLKIQPSEPRDSAVYFCAS

SEQ ID NO: 3 - protein, 95 aa, Artificial
  TCR alpha chain variable  domain of TRAV 8-6
AQSVTQLDSQVPVFEEAPVELRCNYSSSVSVYLFWYVQYPNQGLQLLLKYLSGVSTLVESINGFEAEFNKSQTSFHLRKPSVHISDTAEYFCAVS

SEQ ID NO: 4 - protein, 95 aa, Artificial
  TCR beta chain variable domain of TRBV 6-5
NAGVTQTPKFQVLKTGQSMTLQCAQDMNHEYMSWYRQDPGMGLRLIHYSVGAGITDQGEVPNGYNVSRSTTEDFPLRLLSAAPSQTSVYFCASSY